European Patent Application EP 4 778 391 A1, published July 22, 2026. Title: Method for Preventing Fish Pathogenic Bacteria of Bacteroidota. Applicant: National Institute of Advanced Industrial Science and Technology. The sequence listing filed with the application follows.

SEQUENCE LISTING (16 sequences)

SEQ ID NO: 1 - DNA, 20 bp, synthetic construct
  source 1..20: mol_type = other DNA
agagtttgatcmtggctcag

SEQ ID NO: 2 - DNA, 19 bp, synthetic construct
  source 1..19: mol_type = other DNA
gtgccagcmgccgcggtaa

SEQ ID NO: 3 - DNA, 20 bp, synthetic construct
  source 1..20: mol_type = other DNA
ggactachvgggtwtctaat

SEQ ID NO: 4 - DNA, 22 bp, synthetic construct
  source 1..22: mol_type = other DNA
tacgghtaccttgttacgactt

SEQ ID NO: 5 - DNA, 1386 bp, Peredibacter starrii
  source 1..1386: mol_type = genomic DNA
aacgaacgctggcggcgtgcctaatacatgcaagtcgaacgtgaaaaggggcaacccttagtaaagtggcgcacgggtgagtaacacgtaggtaatctgcctttcagtggggaataacttagggaaacctgagctaatgccgcatacgttagtaataagaaagtgggcgccgcaagggctcatgctgaaagaagggcctgcggcctattagctagttggtggggtaatggcctaccaaggcaacgataggtatccggtctgagaggatgatcggacacactggaactgagacacggtccagactcctacgggaggcagcagtagggaatattgcgcaatgggggaaaccctgacgcagcaacgccgcgtgagtgaggaaggtcttcggattgtaaaactctttttttagggaaaaatgattacagagctaataccctgtaaagtgatggtacctaaagaataagcaccggctaacttcgtgccagcagccgcggtaatacgaagggtgcaagcgttgttcggaatcattgggcgtaaagcgcgcgcaggcggatcagcaagtcagatgtgaaatctcgaagctcaacttcgaaactgcgtctgaaactgctagtctagaatgtcggagggggcaggggaatttcacgtgtaggggtaaaatccgtagagatgtgaaggaacaccggaggcgaaggcgcctgcctggacgactattgacgctgaggcgcgaaagcgtggggagcaaacaggattagataccctggtagtccacgccgtaaacgatgaatactagttattgggggtattgactccttcagtgacgcagctaacgcattaagtattccgcctggggagtacggtcgcaagactaaaactcaaacaaattgacgggggcccgcacaagcggtggattatgtggtttaattcgaagcaacgcgcagaaccttacctaggcttgaactcctacgaacccgttgtaatggacggggtgcccgcaagggaatgtagtgagaggtgctgcatggctgtcgtcagctcgtgttgtgaaatgttgggttaagtctcgcaacgagcgcaacccctatcgtctgttgccagcattaagttgggcactctgacgagactgcctgggttaaccaggaggaaggtggggatgacgtcaagtcctcatggcccttatgtctagggctacacacgtaatacaatggcgcgtacagagggaagcgaactcgcaagggggagcaaatctcaaaaagcgcgcctcagttcggattggagtctgcaactcgactccatgaagttggaatcgctagtaatcggagatcagcacgctccggtgaatacgttcccgggccttgtacacaccgcccgtcacaccatgggagt

SEQ ID NO: 6 - DNA, 1394 bp, Bacteriovoracaceae
  source 1..1394: mol_type = genomic DNA
actcccatggtgtgacgggcggtgtgtacaaggcccgggaacgtattcaccggagcgtgctgatctccgattactagcgattccaacttcatggagtcgagttgcagactccaatccggactgagacgcgctttttgagatttgctccccctcgcgagttcgcttccctctgtacgcgccattgtattacgtgtgtagccctagacataagggccatgaggacttgacgtcatccctaccttcctcctggttaacccaggcagtctcgtcagagtgcccaacttaatgctggcaacagacgataggggttgcgctcgttgcgagacttaacccaacatttcacaacacgagctgacgacagccatgcagcacctctcactacatttccttgcggacactccaggcattaccccggattcgtaggagttcaagcctaggtaaggttctgcgcgttgcttcgaattaaaccacataatccaccgcttgtgcgggcccccgtcaatttgtttgagttttagtcttgcgaccgtacttcccaggcggagcacttaatgcgttagctgcgtcactggaggagtcaatacctccaataactagtgctcatcgtttacggcgtggactaccagggtatctaatcctgtttgctccccacgctttcgcgcctcagcgtcaatgatcatccaggtaggcgccttcgcctccggtgttccttcacatctctacggattttacccctacacgtgaaattcccctaccccctctgatattctagactagtagtttcaggcgcagtttcgaagttgagcttcgagatttcacacctgacttactgatccgcctgcgcgcgctttacgcccaataaatccgaacaacgcttggacccttcgtattaccgcggctgctggcacgaagttagccggtcctttctccttagataccatcacttccaagagatattagctcctgaatcatttttctctaagaacagagttttacaatccgaagaccttcctcactcacgcggcgttgctgcgtcagggtttcccccattgcgcaatattccctactgctgcctcccgtaggagtctggaccgtgtctcagttccagtgtgtccgatcatcctctcagaccggatacctatcgttgccttggtaggccattaccccaccaactagctaataggccgcaggctcttcttttagcgatagcttataaatagaggccatctttgtaatctcttacacatgcggcattagcacaaatttctctgtgttattccccactaaaaggcagatacctacgtgttactcacccgtgcgccactttactcatcccgaaggactttcacgttcgacttgcatgtattaggcacgccgccagcgttcgttctgag

SEQ ID NO: 7 - DNA, 1422 bp, Bacteriovoracaceae
  source 1..1422: mol_type = genomic DNA
tagacgctctcctccttgcggttagagtcacgtcttaaaatgaaaacaactcccatggtgtgacgggcggtgtgtacaaggcccgggaacgtattcaccggagcgtgctgatctccgattactagcgattccaacttcatggagtcgagttgcagactccaatccggactgagacgcgctttttgagatttgctccccctcgcgagttcgcttccctctgtacgcgccattgtattacgtgtgtagccctagacataagggccatgaggacttgacgtcatccctaccttcctcctggttaacccaggcagtctcgtcagagtgcccaacttaatgctggcaacagacgataggggttgcgctcgttgcgagacttaacccaacatttcacaacacgagctgacgacagccatgcagcacctctcactacatttccttgcggacactccaggcattaccccggattcgtaggagttcaagcctaggtaaggttctgcgcgttgcttcgaattaaaccacataatccaccgcttgtgcgggcccccgtcaatttgtttgagttttagtcttgcgaccgtacttcccaggcggagcacttaatgcgttagctgcgtcactggaggagtcaatacctccaataactagtgctcatcgtttacggcgtggactaccagggtatctaatcctgtttgctccccacgctttcgcgcctcagcgtcaatgatcatccaggtaggcgccttcgcctccggtgttccttcacatctctacggattttacccctacacgtgaaattcccctaccccctctgatattctagactagtagtttcaggcgcagtttcgaagttgagcttcgagatttcacacctgacttactgatccgcctgcgcgcgctttacgcccaataaatccgaacaacgcttggacccttcgtattaccgcggctgctggcacctaagttagccggtcctttctccttagataccatcacttccaagagatattagctcctgaatcatttttctctaagaacagagttttacaatccgaagaccttcctcactcacgcggcgttgctgcgtcagggtttcccccattgcgcaatattccctactgctgcctcccgtaggagtctggaccgtgtctcagttccagtgtgtccgatcatcctctcagaccggatacctatcgttgccttggtaggccattaccccaccaactagctaataggccgcaggctcttcttttagcgatagcttataaatagaggccatctttgtaatctcttacacatgcggcattagcacaaatttctctgtggtattccccactaaaaggcagatacctacgtgttactcacccgtgcgccactttactcatcccgaaggactttcacgttcgacttgcatgtattaggcac

SEQ ID NO: 8 - DNA, 1378 bp, Bacteriovoracaceae
  source 1..1378: mol_type = genomic DNA
acgggcggtgtgtacaaggcccgggaacgtattcaccggagcgtgctgatctccgattactagcgattccaacttcatggagtcgagttgcagactccaatccgaactgaggcgcgctttttgagatttgctcccccttgcgagttcgcttccctctgtacgcgccattgtattacgtgtgtagccctagacataagggccatgaggacttgacgtcatccccaccttcctcctggttaacccaggcagtctcgtcagagtgcccaacttaatgctggcaacagacgataggggttgcgctcgttgcgagacttaacccaacatttcacaacacgagctgacgacagccatgcagcacctctcacttcatttccttgcggacactccaggcattaccccggattcgaaggagttcaagcctaggtaaggttctgcgcgttgcttcgaattaaaccacataatccaccgcttgtgcgggcccccgtcaatttgtttgagttttagtcttgcgaccgtactccccaggcggaacacttaatgcgttagctgcgtcactgaaggagtcaatacctccaataactagtgttcatcgtttacggcgtggactaccagggtatctaatcctgtttgctccccacgctttcgcgcctcagcgtcaatagtcgtccaggcaggcgccttcgcctccggtgttccttcacatctctacggattttacccctacacgtgaaattcccctgccccctccgacattctagactagtagtttcaggcgcagtttcggagttgagctccgagatttcacacctgacttactgatccgcctgcgcgcgctttacgcccaatgattccgaacaacgcttgcacccttcgtattaccgcggctgctggcacgaagttagccggtgcttattcctttggtaccatcacttactacgggtattaaccgtaatatcatttttcccaaataaaagagttttacaatccgaagaccttcctcactcacgcggcgttgctgcgtcagggtttcccccattgcgcaatattccctactgctgcctcccgtaggagtctggaccgtgtctcagttccagtgtgtccgatcatcctctcagaccggatacctatcgttgccttggtagtccattacaccaccaactagctaataggccgcaggctcttctttcagcatgagcccttgcggcgcccactttctaattacttacttatgcggcattagcacaactttcgctgtgttattccccactaaaaggcagatgacctacgtgttactcacccgtgcgccactttactcatcccgaaggactttcacgttcgacttgcatgtattaggcacgccgccagcgttcgttctgag

SEQ ID NO: 9 - DNA, 1496 bp, unidentified
  source 1..1496: mol_type = genomic DNA
agtttgatcctggctcagaacgaacgctggcggcgtgcctaatacatgcaagtcgaacgtgaaagtacttcggtatgagtaaagtggcgcacgggtgagtaacacgtaggtaatctgccttatagtggggaacaacttagggaaacctgagctaataccgcatacggaagaaattcgaaaggaggcgtccgcaaggagctttcgctgtaagaagagcctgcgtcctattagctagttggtggggtaatggcctaccaaggctacgataggtatccggtctgagaggatgatcggacacactggaactgagacacggtccagactcctacgggaggcagcagtagggaatattgcgcaatgggggaaaccctgacgcagcaacgccgcgtgagtgaggaaggtcttcggattgtaaaactcttttcttagggaaaaatggttacggagctaataccccgtagtttgatggtacctaaggaataagcaccggctaacttcgtgccagcagccgcggtaatacgaagggtgcaagcgttgttcggaatcattgggcgtaaagcgcgcgcaggcggattgataagtcaggtgtgaaatctcgaagctcaacttcgaaactgcgcctgaaactattagtctagaatgtcggagggggcaggggaatttcacgtgtaggggtaaaatccgtagagatgtgaaggaacaccggaggcgaaggcgcctgcctggacgactattgacgctgaggcgcgaaagcgtggggagcaaacaggattagataccctggtagtccacgccgtaaacgatgagcactagttattggaggtattgactccttcagtgacgcagctaacgcattaagtgctccgcctggggagtacggtcgcaagactaaaactcaaaccaattgacgggggcccgcacaagcggtggattatgtggtttaattcgaagcaacgcgcagaaccttacctaggcttgaactcctccgaatccggggtaatgcctggagtgtccgcaaggaaatggagtgagaggtgctgcatggctgtcgtcagctcgtgttgtgaaatgttgggttaagtctcgcaacgagcgcaacccctatcgtctgttgccagcattaagttgggcactctgacgagactgcctgggttaaccaggaggaaggtggggatgacgtcaagtcctcatggcccttatgtctagggctacacacgtaatacaatggcgcgtacaaagggaagcgaactcgcgagggggagcaaatctcaaaaagcgcgcctcagttcggattggagtctgcaactcgactccatgaagttggaatcgctagtaatcggagatcagcacgctccggtgaatacgttcccgggccttgtacacaccgcccgtcacaccatgggagttgttttcattttaagacgtgactctaaccgcaaggaggagagcgtctacagtgggagcgatgactggggtgaagtcgtaacaaggtaacc

SEQ ID NO: 10 - DNA, 1536 bp, unidentified
  source 1..1536: mol_type = genomic DNA
atcgcccttagagttcgatcctggctcagaacgaacgctggcggcgtgcctaatacatgcaagtcgaacgtgaaaaggggcaacccttagtaaagtggcgcacgggtgagtaacacgtaggtaatctgccttttagtggggaataacttagggaaacctgagctaatgccgcataagtaagtaattagaaaggtggcgtccgcaaggagctaccgctgaaagaagagcctgcggcctattagcttgttggtggggtaatggcctaccaaggcaacgataggtatccggtctgagaggatgatcggacacactggaactgagacacggtccagactcctacgggaggcagcagtagggaatattgcgcaatgggggaaaccctgacgcagcaacgccgcgtgagtgaggaaggtcttcggattgtaaaactcttttgttagggaaaaatggaccagtaactaatagcgctggttttgatggtacctaaagaataagcaccggctaacttcgtgccagcagccgcggtaatacgaagggtgcaagcgttgttcggaattattgggcgtaaagcgcgcgcaggcggatcagcaagtcagatgtgaaatctcgaagctcaacttcgaaactgcgtctgaaactgctagtctagaatgtcggagggggcaggggaatttcacgtgtaggggtaaaatccgtagagatgtgaaggaacaccggaggcgaaggcgcctgcctggacgactattgacgctgaggcgcgaaagcgtggggagcaaacaggattagataccctggtagtccacgccgtaaacgatgagaactagttattgggggtattgactccctcagtgacgcagctaacgcattaagttctccgcctggggagtacggtcgcaagactaaaactcaaacaaattgacgggggcccgcacaagcggtggattatgtggtttaattcgaagcaacgcgcagaaccttacctaggcttgaactcctacgaatccggggtaatgcctggagtgtccgcaaggaaatgtagtgagaggtgctgcatggctgtcgtcagctcgtgttgtgaaatgttgggttaagtctcgcaacgagcgcaacccctatcgtctgttgccagcattaagttgggcactctggcgagactgcctgggttaaccaggaggaaggtggggatgacgtcaagtcctcatggcccttatgtctagggctacacacgtaatacaatggcgcgtacagagggaagcgaactcgcaagggggagcaaatctcaaaaagcgcgcctcagttcggattggagtctgcaactcgactccatgaagttggaatcgctagtaatcggagatcagcacgctccggtgaatacgttcccgggccttgtacacaccgcccgtcacaccatgggagttgttttcattttaagacgtgactctaaccgcaaggaggagagcgtctacagtgggagcgatgactggggtgaagtcgtaacaaggtagccgtaggggaacctgcggctggatcacctcc

SEQ ID NO: 11 - DNA, 1504 bp, unidentified
  source 1..1504: mol_type = genomic DNA
agtttgatcctggctcagaacgaacgctggcggcgtgcctaatacatgcaagtcgaacgtgaaagtacttcggtatgagtaaagtggcgcacgggtgagtaacacgtaggtaatctgccttatagtggggaacaacttagggaaacctgagctaataccgcatacggaagaaattcgaaaggaggcgtccgcaaggagctttcgctgtaagaagagcctgcgtcctattagctagttggtggggtaatggcctaccaaggctacgataggtatccggtctgagaggatgatcggacacactggaactgagacacggtccagactcctacgggaggcagcagtagggaatattgcgcaatgggggaaaccctgacgcagcaacgccgcgtgagtgaggaaggtcttcggattgtaaaactcttttcttagggaaaaatggttaccgggagctaatacccccgtagtttgatgggtacctaagggaataaggcaccggctaacttcgtgccagcagccgcggtaatacgaagggtgcaagcgttgttcggaatcattgggcgtaaagcgcgcgcaggcggattgataagtcaggtgtgaaatctcgaagctcaacttcgaaactgcgcctgaaactattagtctagaatgtcggagggggcaggggaatttcacgtgtaggggtaaaatccgtagagatgtgaaggaacaccggaggcgaaggcgcctgcctggacgactattgacgctgaggcgcgaaagcgtggggagcaaacaggattagataccctggtagtccacgccgtaaacgatgagcactagttattggaggtattgactccttcagtgacgcagctaacgcattaagtgctccgcctggggagtacggtcgcaagactaaaactcaaacaaattgacgggggcccgcacaagcggtggattatgtggtttaattcgaagcaacgcgcagaaccttacctaggcttgaactcctccgaatccgggttaatgcctggagtgatccgcaaggaaatggatttcgcgttgctgcgatggctgtcgtcagctcgtgttgtgaaatgttgggttaagtctcgcaacgagcgcaacccctatcgtctgttgccagcattaagttgggcactctgacgagactgcctgggttaaccaggaggaaggtggggatgacgtcaagtcctcatggcccttatgtctagggctacacacgtaatacaatggcgcgtacaaagggaagcgaactcgcgagggggagcaaatctcaaaaagcgcgcctcagttcggattggagtctgcaactcgactccatgaagttggaatcgctagtaatcggagatcagcacgctccggtgaatacgttcccgggccttgtacacaccgcccgtcacaccatgggagttgttttcattttaagacgtgactctaaccgcaaggaggagagcgtctacagtgggagcgatgactggggtgaagtcgtaacaaggtaacc

SEQ ID NO: 12 - DNA, 1392 bp, Peredibacter starrii
  source 1..1392: mol_type = genomic DNA
ctcagaacgaacgctggcggcgtgcctaaatacatgcaagtcgaacgtgaaaaggggcaacccttagtaaagtggcgcacgggtgagtaacacgtaggtaatctgcctttcagtggggaataacttagggaaacctgagctaatgccgcatacgttagtaataagaaagtgggcgccgcaagggctcatgctgaaagaagggcctgcggcctattagctagttggtggggtaatggcctaccaaggcaacgataggtatccggtctgagaggatgatcggacacactggaactgagacacggtccagactcctacgggaggcagcagtagggaatattgcgcaatgggggaaaccctgacgcagcaacgccgcgtgagtgaggaaggtcttcggattgtaaaactctttttttagggaaaaatgattacagagctaataccctgtaaagtgatggtacctaaagaataagcaccggctaacttcgtgccagcagccgcggtaatacgaagggtgcaagcgttgttcggaatcattgggcgtaaagcgcgcgcaggcggatcagcaagtcagatgtgaaatctcgaagctcaacttcgaaactgcgtctgaaactgctagtctagaatgtcggagggggcaggggaatttcacgtgtaggggtaaaatccgtagagatgtgaaggaacaccggaggcgaaggcgcctgcctggacgactattgacgctgaggcgcgaaagcgtggggagcaaacaggattagataccctggtagtccacgccgtaaacgatgaatactagttattgggggtattgactccttcagtgacgcagctaacgcattaagtattccgcctggggagtacggtcgcaagactaaaactcaaacaaattgacgggggcccgcacaagcggtggattatgtggtttaattcgaagcaacgcgcagaaccttacctaggcttgaactcctacgaacccgttgtaatggacggggtgcccgcaagggaatgtagtgagaggtgctgcatggctgtcgtcagctcgtgttgtgaaatgttgggttaagtctcgcaacgagcgcaacccctatcgtctgttgccagcattaagttgggcactctgacgagactgcctgggttaaccaggaggaaggtggggatgacgtcaagtcctcatggcccttatgtctagggctacacacgtaatacaatggcgcgtacagagggaagcgaactcgcaagggggagcaaatctcaaaaagcgcgcctcagttcggattggagtctgcaactcgactccatgaagttggaatcgctagtaatcggagatcagcacgctccggtgaatacgttcccgggccttgtacacaccgcccgtcacaccatgggagt

SEQ ID NO: 13 - DNA, 1513 bp, unidentified
  source 1..1513: mol_type = genomic DNA
agtttgatcctggctcagaacgaacgctggcggcgtgcctaatacatgcaagtcgaacgtgaaagtacttcggtatgagtaaagtggcgcacgggtgagtaacacgtaggtaatctgccttatagtggggaacaacttagggaaacctgagctaataccgcatacggaagaaattcgaaaggaggcgtccgcaaggagctttcgctgtaagaagagcctgcgtcctattagctagttggtggggtaatggcctaccaaggctacgataggtatccggtctgagaggatgatcggacacactggaactgagacacggtccagactcctacgggaggcagcagtagggaatattgcgcaatgggggaaaccctgacgcagcaacgccgcgtgagtgaggaaggtcttcggattgtaaaactcttttcttagggaaaaatggttacggagctaataccccgtagtttgatggtacctaaggaataagcaccggctaacttcgtgccagcagccgcggtaatacgaagggtgcaagcgttgttcggaatcattgggcgtaaagcgcgcgcaggcggattgataagtcaggtgtgaaatctcgaagctcaacttcgaaactgcgcctgaaactattagtctagaatgtcggaagggggcaggggaattttcacgtgtaggggtaaaatccgtagagatgtgaaggaacaccggaggcgaaggcgcctgcctggacgactattgacgctgaggcgcgaaagcgtggggagcaaacaggattagataccctggtagtccacgccgtaaacgatgagcactagttattggaggtattgactccttcagtgacgcagctaacgcattaagtgctccgcctggggagtacggtcgcaagactaaaactcaaacaaattgacgggggcccgcacaagcggtggattatgtggtttaaactcaaagcaaattgaccgcgcagaaccttacctaggcttgaactcctccgaatccggggtaatgcctggagtgtccgcaaggaaatggagtgagaggtgctgcatggctgtcgtcagctcgtgttgtgaaatgttgggttaagtctcgcaacgagcgcaacccctatcgtctgttgccagcattaagttgggcactctgaacgagactgccttgggttaaaccaggaaggaaggtggggaatgacgtcaagtcctcatggccctttatgtctagggcttacacacgtaatacaatggcgcgtacaaagggaagcgaactcgcgaggggggagcaaatctcaaaaagcgcgcctcagttcggattggagtctgcaactcgactccatgaagttggaatcgctagtaatcggaaatcagcacgctccggggaatacgttcccgggccttgtacacaccgcccgtcacaccatgggagttgttttcattttaagacgtgactctaaccgcaaggaggagagcgtctacagtgggagcgatgactggggtgaagtcgtaacaaggtaacc

SEQ ID NO: 14 - DNA, 1460 bp, unidentified
  source 1..1460: mol_type = genomic DNA
aacgaacgctggcggcgtgcctaatacatgcaagtcgagcgagaaagtccttcgggatgagtacagcggcgcacgggtgagtaacacgtaggtacctgccctttagtggggaacaacaccgggaaaccggtgctaataccgcataagtaggaaactagaaagatggcctctatttataagctatcgctaaaggaagggcctgcgctgcattagctagttggtggggtaatggcctaccaaggccacgatgcatatccggtctgagaggatgatcggacacactggaactgagacacggtccagactcctacgggaggcagcagtagggaatattgcgcaatgggggaaaccctgacgcagcaacgccgcgtgagtgaggaaggtcttcggattgtaaaactcttttcttagagaaaaatgtccatatggctaatatccatgcggagtgatggtatctaaggaataagcaccggctaacttcgtgccagcagccgcggtaatacgaagggtgcaagcgttgttcggaatcattgggcgtaaagcgcgcgcaggcggatcagtaagtcaggtgtgaaatctcggagctcgactccgaaactgcgcctgaaactactagtctagaatgtcggagggggcaggggaatttcacgtgtaggggtaaaatccgtagagatgtgaaggaacaccggaggcgaaggcgcctgcctggacgactattgacgctgaggcgcgaaagcgtggggagcaaacaggattagataccctggtagtccacgccgtaaacgatgagcactagttattaggggtattgactcccttggtgacgcagctaacgcattaagtgctccgcctgggaagtacggtcgcaagactaaaactcaaacaaattgacgggggcccgcacaagcggtggattatgtggtttaattcgaagcaacgcgcagaaccttacctaggcttgaactcctctgaatccggggtaatgcctggagtgtccgcaaggaaatagagtgagaggtgctgcatgactgtcgtcagctcgtgttgtgaaatgttgggttaagtctcgcaacgagcgcaacccctatcatcagttgccagcattaagttgggcactctgatgagactgcctgggttaaccaggaggaaggtggggatgacgtcaagtcctcatggcccttatgtctagggctacacacgtaatacaatggcgcgtacagagggaagcgaaccagcgatggggagcaaatctcaaaaagcgcgtctcagtccggattgaagtctgcaactcgacttcatgaagttggaatcgctagtaatcggagatcagcacgctccggtgaatacgttcccgggccttgtacacaccgcccgtcacaccatgggagttgttttcattttaagacgtgactctaaccgcaaggaggagagcgtctacagtgggagcgatgactggggtg

SEQ ID NO: 15 - DNA, 1361 bp, unidentified
  source 1..1361: mol_type = genomic DNA
acgggcggtgtgtacaaggcccgggaacgtattcaccggagcgtgctgatctccgattactagcgattccaacttcatggagtcgagttgcagactccaatccgnactgagncgcgctttttgagatttgctccccctngcgagttcgcttccctctgtacgcgccattgtattacgtgtgtagccctagacataagggccatgaggacttgacgtcatcccnaccttcctcctggttaacccaggcagtctcgtcagagtgcccaacttaatgctggcaacagacgataggggttgcgctcgttgcgagacttaacccaacatttcacaacacgagctgacgacagccatgcagcacctctcactncatttccttgcggacactccaggcattaccccggattcgnaggagttcaagcctaggtaaggttctgcgcgttgcttcgaattaaaccacataatccaccgcttgtgcgggcccccgtcaatttgtttgagttttagtcttgcgaccgtactncccaggcggancacttaatgcgttagctgcgtcactgnaggagtcaatacctccaataactagtgntcatcgtttacggcgtggactaccagggtatctaatcctgtttgctccccacgctttcgcgcctcagcgtcaatnntcntccaggnaggcgccttcgcctccggtgttccttcacatctctacggattttacccctacacgtgaaattcccctnccccctcnganattctagactagtagtttcaggcgcagtttcgnagttgagctncgagatttcacacctgacttactgatccgcctgcgcgcgctttacgcccaatnantccgaacaacgcttgnacccttcgtattaccgcggctgctggcancnaagttagccggtncttnntccttngntaccatcacttncnanngntattancnnnnnnatcatttttcncnaanaanagagttttacaatccgaagaccttcctcactcacgcggcgttgctgcgtcagggtttcccccattgcgcaatattccctactgctgcctcccgtaggagtctggaccgtgtctcagttccagtgtgtccgatcatcctctcagaccggatacctatcgttgccttggtagnccattacnccaccaactagctaataggccgcaggctcttctttnagcnnnagcnnntnnnnngnngccnnctttntaatnncttacnnatgcggcattagcacaantttcnctgtgntattccccactaaaaggcagatnacctacgtgttactcacccgtgcgccactttactcatcccgaaggactttcacgttcgacttgcatgtattaggcac

SEQ ID NO: 16 - DNA, 1461 bp, unidentified
  source 1..1461: mol_type = genomic DNA
aacgaacgctggcggcgtgcctaatacatgcaagtcgaacgtgaaagtccttcgggatgagtaaagtggcgcacgggtgagtaacacgtaggtaatctgcctttcagtggggaataacttcgggaaaccggagctaatgccgcatacgtaagtaattagaaagaaggcctctatttataagctttcgctgagagaagagcctgcgtcctattagctagttggtagggtaaaagcctaccaaggcaacgataggtatccggtctgagaggatgatcggacacactggaactgagacacggtccagactcctacgggaggcagcagtagggaatattgcgcaatgggggaaaccctgacgcagcaacgccgcgtgagtgaggaaggtcttaggattgtaaaactcttttatttgggaaaaatgaccatatggctaatatccatgtggagtgatggtaccaaaggaataagcaccggctaacttcgtgccagcagccgcggtaatacgaagggtgcaagcgttgttcggaatcattgggcgtaaagcgcgcgcaggcggatcagcaagtcagatgtgaaatctcgaagctcaacttcgaaactgcgtctgaaactgctagtctagaatgtcggagggggcaggggaatttcacgtgtaggggtaaaatccgtagagatgtgaaggaacaccggaggcgaaggcgcctgcctggacgactattgacgctgaggcgcgaaagcgtggggagcaaacaggattagataccctggtagtccacgccgtaaacgatgagcactagttattgggggtattgactccctcagtgacgcagctaacgcattaagtgctccgcctgggaagtacggtcgcaagactaaaactcaaacaaattgacgggggcccgcacaagcggtggactatgtggtttaattcgaagcaacgcgcagaaccttacctaggcttgaactcctacgaatccggggtaatgcctggagtgtccgcaaggaaatgtagtgagaggtgctgcaaggctgtcgtcagctcgtgttgtgaaatgttgggttaagtctcgcaacgagcgcaacccctatcgtctgttgccagcattaagttgggcactctgacgagactgcctgggttaaccaggaggaaggtggggatgacgtcaagtcctcatggcccttatgtctagggctacacacgtaatacaatggcgcgtacagagggaagcgaaccagcgatggggagcaaatctcaaaaagcgcgcctcagttcggattggagtctgcaactcgactccatgaagttggaatcgctagtaatcggagatcagcacgctccggtgaatacgttcccgggccttgtacacaccgcccgtcacaccatgggagtgggctgcaaaagaagtgggtagtttaaccttcgggaggacgctcaccactttgtggttcatgactggggtg